European Patent Application EP 4 534 566 A1, published April 9, 2025. Title: HYALURONIC ACID DERIVATIVE, PHARMACEUTICAL COMPOSITION, AND METHOD OF PRODUCING PHARMACEUTICAL COMPOSITION. Applicant: Asahi Kasei Corporation. The sequence listing filed with the application follows.

SEQUENCE LISTING (5 sequences)

SEQ ID NO: 1 - protein, 37 aa, synthetic construct
NDHIAYFLYQILRGLQYIHSANVLHRDLKPSNLLLNT

SEQ ID NO: 2 - protein, 38 aa, synthetic construct
SVYDFFVWLYYYYYYTWHRYHLLYYYYYYEGSRNQDWL

SEQ ID NO: 3 - protein, 40 aa, synthetic construct
GSNPARYEFLWGPRALAETSYVKVLEHVVRVNARVRIAYP

SEQ ID NO: 4 - protein, 9 aa, synthetic construct
QYIHSANVL

SEQ ID NO: 5 - protein, 17 aa, synthetic construct
RGLQYIHSANVLHRDLK